European Patent Application EP 4 621 058 A1, published September 24, 2025. Title: IMMUNOENHANCING SALMONELLA STRAIN FOR TREATMENT OF CANCER AND USE THEREOF. Applicant: CNCure Co., Ltd. Application KR 10-2022-0151641, filed November 14, 2022. The sequence listing filed with the application follows.

SEQUENCE LISTING (3 sequences)

SEQ ID NO: 1 - DNA, 348 bp, Homo sapiens
  source 1..348: mol_type = genomic DNA
atgaattgggtcaacgtgattagcgatctgaaaaagatcgaagatctcattcagagcatgcatattgatgctacgctgtatacagaatccgacgtgcatccgagctgcaaagttactgcaatgaagtgcttcctgctggaactgcaggtaataagcctggagagcggtgacgcgagcatccatgatacagttgaaaatctgataatcctggcaaacaactcgctgagcagcaatggtaatgtgacggaatcaggctgcaaagaatgtgaggagctggaagaaaaaaacatcaaagagttcctgcagagcttcgtccacattgttcaaatgtttattaacaccagctaa

SEQ ID NO: 2 - DNA, 345 bp, Mus musculus
  source 1..345: mol_type = genomic DNA
atgaattggatcgatgtacgctatgacctggaaaaaattgaatcactgattcagagcattcatatcgacactaccctgtataccgatagcgattttcatccgtcctgcaaagtgacagcaatgaactgtttcctgctcgaactgcaggtcattctgcacgagtatagcaatatgaccctgaacgagacggtgcgtaatgttctgtacctggcgaatagcaccctgagcagcaataaaaacgttgctgaaagcggatgtaaagaatgcgaggaactcgaggaaaagacgtttactgaatttctgcagagcttcattcggatagtccaaatgttcattaacacgtca

SEQ ID NO: 3 - DNA, 66 bp, synthetic construct
  source 1..66: mol_type = other DNA
atgaaatacctattgcctacggcagccgctggattgttattactcgcggcccaaccggccatggcc